European Patent Application EP 4 261 281 A1, published October 18, 2023. Title: Modified polypeptide having xylanase activity. Applicant: CJ CheilJedang Corporation. The sequence listing filed with the application follows.

SEQUENCE LISTING (36 sequences)

SEQ ID NO: 1 - protein, 227 aa, Artificial Sequence
  Op Xyn
GQRLSVGGGQNQHKGVFDGFSYEIWLDNTGGSGSMTLGKGATFKAEWSAAVNRGNFLARRGLDFGSTKKATAYEYIGLDYEASYRQTASASGNSRLCVYGWFQNRGVQGVPLVEYYIIEDWVDWVPDAQGKMVTIDGAQYKIFQMDHTGPTINGGNETFKQYFSVRQQKRTSGHITVSDHFKAWANQGWGIGNLYEVTLNAEGWQSSGVADVTKLDVYTTKQGSAPR

SEQ ID NO: 2 - DNA, 684 bp, Artificial Sequence
  Op Xyn nt
ggccagaggttgagcgtcggtggtggccagaaccagcacaagggcgtcttcgatggcttcagctacgagatctggctggataacaccggcggtagcggttccatgaccctgggtaagggagctaccttcaaggctgagtggagcgcagctgtcaaccggggtaacttcctggcccgacgcggtctggatttcggctccaccaagaaggccaccgcttacgagtacatcggcctggattacgaggcaagctacaggcagactgccagcgcaagcggtaacagccgcctctgcgtctacggctggttccagaaccggggagtgcagggcgtccccctggtcgagtactacatcatcgaggattgggtcgactgggtcccggatgcgcagggaaagatggtcaccatcgatggcgcccagtacaagatcttccagatggatcacactggcccgaccatcaacggcggtaacgagaccttcaagcagtacttcagcgtccgccagcagaagcgcactagcggccacatcaccgtcagcgatcacttcaaggcgtgggccaaccagggctggggcatcggcaacctctacgaggtcacactgaacgcagagggttggcagagcagtggtgtcgccgacgtcaccaagctggatgtctacaccaccaagcagggttcggcccctcgttag

SEQ ID NO: 3 - protein, 227 aa, Artificial Sequence
  DS1(R3C+T36C)
GQCLSVGGGQNQHKGVFDGFSYEIWLDNTGGSGSMCLGKGATFKAEWSAAVNRGNFLARRGLDFGSTKKATAYEYIGLDYEASYRQTASASGNSRLCVYGWFQNRGVQGVPLVEYYIIEDWVDWVPDAQGKMVTIDGAQYKIFQMDHTGPTINGGNETFKQYFSVRQQKRTSGHITVSDHFKAWANQGWGIGNLYEVTLNAEGWQSSGVADVTKLDVYTTKQGSAPR

SEQ ID NO: 4 - DNA, 684 bp, Artificial Sequence
  DS1(R3C+T36C) nt
ggccagtgtttgagcgtcggtggtggccagaaccagcacaagggcgtcttcgatggcttcagctacgagatctggctggataacaccggcggtagcggttccatgtgtctgggtaagggagctaccttcaaggctgagtggagcgcagctgtcaaccggggtaacttcctggcccgacgcggtctggatttcggctccaccaagaaggccaccgcttacgagtacatcggcctggattacgaggcaagctacaggcagactgccagcgcaagcggtaacagccgcctctgcgtctacggctggttccagaaccggggagtgcagggcgtccccctggtcgagtactacatcatcgaggattgggtcgactgggtcccggatgcgcagggaaagatggtcaccatcgatggcgcccagtacaagatcttccagatggatcacactggcccgaccatcaacggcggtaacgagaccttcaagcagtacttcagcgtccgccagcagaagcgcactagcggccacatcaccgtcagcgatcacttcaaggcgtgggccaaccagggctggggcatcggcaacctctacgaggtcacactgaacgcagagggttggcagagcagtggtgtcgccgacgtcaccaagctggatgtctacaccaccaagcagggttcggcccctcgttag

SEQ ID NO: 5 - protein, 227 aa, Artificial Sequence
  DS2(S5C+S34C)
GQRLCVGGGQNQHKGVFDGFSYEIWLDNTGGSGCMTLGKGATFKAEWSAAVNRGNFLARRGLDFGSTKKATAYEYIGLDYEASYRQTASASGNSRLCVYGWFQNRGVQGVPLVEYYIIEDWVDWVPDAQGKMVTIDGAQYKIFQMDHTGPTINGGNETFKQYFSVRQQKRTSGHITVSDHFKAWANQGWGIGNLYEVTLNAEGWQSSGVADVTKLDVYTTKQGSAPR

SEQ ID NO: 6 - DNA, 684 bp, Artificial Sequence
  DS2(S5C+S34C) nt
ggccagaggttgtgtgtcggtggtggccagaaccagcacaagggcgtcttcgatggcttcagctacgagatctggctggataacaccggcggtagcggttgtatgaccctgggtaagggagctaccttcaaggctgagtggagcgcagctgtcaaccggggtaacttcctggcccgacgcggtctggatttcggctccaccaagaaggccaccgcttacgagtacatcggcctggattacgaggcaagctacaggcagactgccagcgcaagcggtaacagccgcctctgcgtctacggctggttccagaaccggggagtgcagggcgtccccctggtcgagtactacatcatcgaggattgggtcgactgggtcccggatgcgcagggaaagatggtcaccatcgatggcgcccagtacaagatcttccagatggatcacactggcccgaccatcaacggcggtaacgagaccttcaagcagtacttcagcgtccgccagcagaagcgcactagcggccacatcaccgtcagcgatcacttcaaggcgtgggccaaccagggctggggcatcggcaacctctacgaggtcacactgaacgcagagggttggcagagcagtggtgtcgccgacgtcaccaagctggatgtctacaccaccaagcagggttcggcccctcgttag

SEQ ID NO: 7 - protein, 227 aa, Artificial Sequence
  DS5(F20C+A41C)
GQRLSVGGGQNQHKGVFDGCSYEIWLDNTGGSGSMTLGKGCTFKAEWSAAVNRGNFLARRGLDFGSTKKATAYEYIGLDYEASYRQTASASGNSRLCVYGWFQNRGVQGVPLVEYYIIEDWVDWVPDAQGKMVTIDGAQYKIFQMDHTGPTINGGNETFKQYFSVRQQKRTSGHITVSDHFKAWANQGWGIGNLYEVTLNAEGWQSSGVADVTKLDVYTTKQGSAPR

SEQ ID NO: 8 - DNA, 684 bp, Artificial Sequence
  DS5(F20C+A41C) nt
ggccagaggttgagcgtcggtggtggccagaaccagcacaagggcgtcttcgatggctgtagctacgagatctggctggataacaccggcggtagcggttccatgaccctgggtaagggatgtaccttcaaggctgagtggagcgcagctgtcaaccggggtaacttcctggcccgacgcggtctggatttcggctccaccaagaaggccaccgcttacgagtacatcggcctggattacgaggcaagctacaggcagactgccagcgcaagcggtaacagccgcctctgcgtctacggctggttccagaaccggggagtgcagggcgtccccctggtcgagtactacatcatcgaggattgggtcgactgggtcccggatgcgcagggaaagatggtcaccatcgatggcgcccagtacaagatcttccagatggatcacactggcccgaccatcaacggcggtaacgagaccttcaagcagtacttcagcgtccgccagcagaagcgcactagcggccacatcaccgtcagcgatcacttcaaggcgtgggccaaccagggctggggcatcggcaacctctacgaggtcacactgaacgcagagggttggcagagcagtggtgtcgccgacgtcaccaagctggatgtctacaccaccaagcagggttcggcccctcgttag

SEQ ID NO: 9 - DNA, 20 bp, Artificial Sequence
  primer
ggccagtgtttgagcgtcgg

SEQ ID NO: 10 - DNA, 22 bp, Artificial Sequence
  primer
gctcaaacactggcccatatgg

SEQ ID NO: 11 - DNA, 24 bp, Artificial Sequence
  primer
aagggatgtaccttcaaggctgag

SEQ ID NO: 12 - DNA, 24 bp, Artificial Sequence
  primer
acccagacacatggaaccgctacc

SEQ ID NO: 13 - DNA, 20 bp, Artificial Sequence
  primer
aggttgtgtgtcggtggtgg

SEQ ID NO: 14 - DNA, 21 bp, Artificial Sequence
  primer
accgacacacaacctctggcc

SEQ ID NO: 15 - DNA, 24 bp, Artificial Sequence
  primer
agcggttgtatgaccctgggtaag

SEQ ID NO: 16 - DNA, 21 bp, Artificial Sequence
  primer
ggtcatacaaccgctaccgcc

SEQ ID NO: 17 - DNA, 26 bp, Artificial Sequence
  primer
ccggattgtcagggaaagatggtcac

SEQ ID NO: 18 - DNA, 22 bp, Artificial Sequence
  primer
tccctgacaatccgggacccag

SEQ ID NO: 19 - DNA, 26 bp, Artificial Sequence
  primer
aagatctgtcagatggatcacactgg

SEQ ID NO: 20 - DNA, 25 bp, Artificial Sequence
  primer
catctgacagatcttgtactgggcg

SEQ ID NO: 21 - DNA, 21 bp, Artificial Sequence
  primer
ttcggctgtaccaagaaggcc

SEQ ID NO: 22 - DNA, 24 bp, Artificial Sequence
  primer
cttggtacagccgaaatccagacc

SEQ ID NO: 23 - DNA, 24 bp, Artificial Sequence
  primer
atcggctgtctctacgaggtcgca

SEQ ID NO: 24 - DNA, 20 bp, Artificial Sequence
  primer
gtagagacagccgatgcccc

SEQ ID NO: 25 - DNA, 24 bp, Artificial Sequence
  primer
gatggctgtagctacgagatctgg

SEQ ID NO: 26 - DNA, 23 bp, Artificial Sequence
  primer
gtagctacagccatcgaagacgc

SEQ ID NO: 27 - DNA, 24 bp, Artificial Sequence
  primer
aagggatgtaccttcaaggctgag

SEQ ID NO: 28 - DNA, 23 bp, Artificial Sequence
  primer
gaaggtacatcccttacccaggg

SEQ ID NO: 29 - DNA, 25 bp, Artificial Sequence
  primer
aaggcctgtgcttacgagtacatcg

SEQ ID NO: 30 - DNA, 23 bp, Artificial Sequence
  primer
gtaagcacaggccttcttggtgg

SEQ ID NO: 31 - DNA, 22 bp, Artificial Sequence
  primer
tggggctgtggcaacctctacg

SEQ ID NO: 32 - DNA, 19 bp, Artificial Sequence
  primer
gttgccacagccccagccc

SEQ ID NO: 33 - DNA, 23 bp, Artificial Sequence
  primer
cgcggttgtgatttcggctccac

SEQ ID NO: 34 - DNA, 21 bp, Artificial Sequence
  primer
gaaatcacaaccgcgtcgggc

SEQ ID NO: 35 - DNA, 25 bp, Artificial Sequence
  primer
ctggattgttacaccaccaagcagg

SEQ ID NO: 36 - DNA, 25 bp, Artificial Sequence
  primer
ggtgtaacaatccagcttggtgacg